European Patent Specification EP 3 436 605 B1, published June 18, 2025. Title: AMPLIFICATION OF TARGET SEQUENCES. Applicant: Reproductive Health Science Limited. The sequence listing filed with the application follows.

SEQUENCE LISTING (7 sequences)

SEQ ID NO: 1 - DNA, 22 bp, Artificial Sequence
  Primer sequence
aaattttttgccaataaagata

SEQ ID NO: 2 - DNA, 22 bp, Artificial Sequence
  Primer sequence
tctcagcaagctatgagtaggt

SEQ ID NO: 3 - DNA, 24 bp, Artificial Sequence
  Primer sequence
catgaacgcattcatcgtgtggtc

SEQ ID NO: 4 - DNA, 25 bp, Artificial Sequence
  Primer sequence
ctgcgggaagcaaactgcaattctt

SEQ ID NO: 5 - DNA, 16 bp, Artificial Sequence
  Pirmer sequence
  misc_feature (7)..(10): n is a, c, g, or t
ctcgagnnnnatgtgg

SEQ ID NO: 6 - DNA, 21 bp, Artificial Sequence
  Primer sequence
  misc_feature (10)..(15): n is a, c, g, or t
cgactcgagnnnnnnatgtgg

SEQ ID NO: 7 - DNA, 21 bp, Artificial Sequence
  Primer sequence
  misc_feature (10)..(15): n is a, c, g, or t
ccgaccgagnnnnnnatgtgg